European Patent Specification EP 3 600 409 B1, published August 14, 2024. Title: T CELL RECEPTORS AND IMMUNE THERAPY USING THE SAME AGAINST PRAME POSITIVE CANCERS. Applicant: Immatics Biotechnologies GmbH. The sequence listing filed with the application follows.

SEQUENCE LISTING (204 sequences)

SEQ ID NO: 1 - protein, 6 aa, Homo sapiens
SSNFYA

SEQ ID NO: 2 - protein, 3 aa, Homo sapiens
MTL

SEQ ID NO: 3 - protein, 11 aa, Homo sapiens
CALYNNNDMRF

SEQ ID NO: 4 - protein, 132 aa, Homo sapiens
MEKNPLAAPLLILWFHLDCVSSILNVEQSPQSLHVQEGDSTNFTCSFPSSNFYALHWYRWETAKSPEALFVMTLNGDEKKKGRISATLNTKEGYSYLYIKGSQPEDSATYLCALYNNNDMRFGAGTRLTVKP

SEQ ID NO: 5 - protein, 141 aa, Homo sapiens
NIQNPDPAVYQLRDSKSSDKSVCLFTDFDSQTNVSQSKDSDVYITDKTVLDMRSMDFKSNSAVAWSNKSDFACANAFNNSIIPEDTFFPSPESSCDVKLVEKSFETDTNLNFQNLSVIGFRILLLKVAGFNLLMTLRLWSS

SEQ ID NO: 6 - protein, 273 aa, Homo sapiens
MEKNPLAAPLLILWFHLDCVSSILNVEQSPQSLHVQEGDSTNFTCSFPSSNFYALHWYRWETAKSPEALFVMTLNGDEKKKGRISATLNTKEGYSYLYIKGSQPEDSATYLCALYNNNDMRFGAGTRLTVKPNIQNPDPAVYQLRDSKSSDKSVCLFTDFDSQTNVSQSKDSDVYITDKTVLDMRSMDFKSNSAVAWSNKSDFACANAFNNSIIPEDTFFPSPESSCDVKLVEKSFETDTNLNFQNLSVIGFRILLLKVAGFNLLMTLRLWSS

SEQ ID NO: 7 - protein, 5 aa, Homo sapiens
SGHNS

SEQ ID NO: 8 - protein, 6 aa, Homo sapiens
FNNNVP

SEQ ID NO: 9 - protein, 13 aa, Homo sapiens
CASSPGSTDTQYF

SEQ ID NO: 10 - protein, 132 aa, Homo sapiens
MDSWTFCCVSLCILVAKHTDAGVIQSPRHEVTEMGQEVTLRCKPISGHNSLFWYRQTMMRGLELLIYFNNNVPIDDSGMPEDRFSAKMPNASFSTLKIQPSEPRDSAVYFCASSPGSTDTQYFGPGTRLTVL

SEQ ID NO: 11 - protein, 179 aa, Homo sapiens
EDLKNVFPPEVAVFEPSEAEISHTQKATLVCLATGFYPDHVELSWWVNGKEVHSGVSTDPQPLKEQPALNDSRYCLSSRLRVSATFWQNPRNHFRCQVQFYGLSENDEWTQDRAKPVTQIVSAEAWGRADCGFTSESYQQGVLSATILYEILLGKATLYAVLVSALVLMAMVKRKDSRG

SEQ ID NO: 12 - protein, 311 aa, Homo sapiens
MDSWTFCCVSLCILVAKHTDAGVIQSPRHEVTEMGQEVTLRCKPISGHNSLFWYRQTMMRGLELLIYFNNNVPIDDSGMPEDRFSAKMPNASFSTLKIQPSEPRDSAVYFCASSPGSTDTQYFGPGTRLTVLEDLKNVFPPEVAVFEPSEAEISHTQKATLVCLATGFYPDHVELSWWVNGKEVHSGVSTDPQPLKEQPALNDSRYCLSSRLRVSATFWQNPRNHFRCQVQFYGLSENDEWTQDRAKPVTQIVSAEAWGRADCGFTSESYQQGVLSATILYEILLGKATLYAVLVSALVLMAMVKRKDSRG

SEQ ID NO: 13 - protein, 6 aa, Homo sapiens
DRGSQS

SEQ ID NO: 14 - protein, 2 aa, Homo sapiens
IY

SEQ ID NO: 15 - protein, 15 aa, Homo sapiens
CAAVISNFGNEKLTF

SEQ ID NO: 16 - protein, 134 aa, Homo sapiens
MKSLRVLLVILWLQLSWVWSQQKEVEQNSGPLSVPEGAIASLNCTYSDRGSQSFFWYRQYSGKSPELIMFIYSNGDKEDGRFTAQLNKASQYVSLLIRDSQPSDSATYLCAAVISNFGNEKLTFGTGTRLTIIP

SEQ ID NO: 17 - protein, 141 aa, Homo sapiens; identical to SEQ ID NO: 5

SEQ ID NO: 18 - protein, 275 aa, Homo sapiens
MKSLRVLLVILWLQLSWVWSQQKEVEQNSGPLSVPEGAIASLNCTYSDRGSQSFFWYRQYSGKSPELIMFIYSNGDKEDGRFTAQLNKASQYVSLLIRDSQPSDSATYLCAAVISNFGNEKLTFGTGTRLTIIPNIQNPDPAVYQLRDSKSSDKSVCLFTDFDSQTNVSQSKDSDVYITDKTVLDMRSMDFKSNSAVAWSNKSDFACANAFNNSIIPEDTFFPSPESSCDVKLVEKSFETDTNLNFQNLSVIGFRILLLKVAGFNLLMTLRLWSS

SEQ ID NO: 19 - protein, 5 aa, Homo sapiens
SGHRS

SEQ ID NO: 20 - protein, 6 aa, Homo sapiens
YFSETQ

SEQ ID NO: 21 - protein, 14 aa, Homo sapiens
CASSPWDSPNEQYF

SEQ ID NO: 22 - protein, 132 aa, Homo sapiens
MGSRLLCWVLLCLLGAGPVKAGVTQTPRYLIKTRGQQVTLSCSPISGHRSVSWYQQTPGQGLQFLFEYFSETQRNKGNFPGRFSGRQFSNSRSEMNVSTLELGDSALYLCASSPWDSPNEQYFGPGTRLTVT

SEQ ID NO: 23 - protein, 179 aa, Homo sapiens; identical to SEQ ID NO: 11

SEQ ID NO: 24 - protein, 311 aa, Homo sapiens
MGSRLLCWVLLCLLGAGPVKAGVTQTPRYLIKTRGQQVTLSCSPISGHRSVSWYQQTPGQGLQFLFEYFSETQRNKGNFPGRFSGRQFSNSRSEMNVSTLELGDSALYLCASSPWDSPNEQYFGPGTRLTVTEDLKNVFPPEVAVFEPSEAEISHTQKATLVCLATGFYPDHVELSWWVNGKEVHSGVSTDPQPLKEQPALNDSRYCLSSRLRVSATFWQNPRNHFRCQVQFYGLSENDEWTQDRAKPVTQIVSAEAWGRADCGFTSESYQQGVLSATILYEILLGKATLYAVLVSALVLMAMVKRKDSRG

SEQ ID NO: 25 - protein, 6 aa, Homo sapiens
NSAFQY

SEQ ID NO: 26 - protein, 2 aa, Homo sapiens
TY

SEQ ID NO: 27 - protein, 13 aa, Homo sapiens
CAMSEAAGNKLTF

SEQ ID NO: 28 - protein, 133 aa, Homo sapiens
MMKSLRVLLVILWLQLSWVWSQQKEVEQDPGPLSVPEGAIVSLNCTYSNSAFQYFMWYRQYSRKGPELLMYTYSSGNKEDGRFTAQVDKSSKYISLFIRDSQPSDSATYLCAMSEAAGNKLTFGGGTRVLVKP

SEQ ID NO: 29 - protein, 141 aa, Homo sapiens; identical to SEQ ID NO: 5

SEQ ID NO: 30 - protein, 274 aa, Homo sapiens
MMKSLRVLLVILWLQLSWVWSQQKEVEQDPGPLSVPEGAIVSLNCTYSNSAFQYFMWYRQYSRKGPELLMYTYSSGNKEDGRFTAQVDKSSKYISLFIRDSQPSDSATYLCAMSEAAGNKLTFGGGTRVLVKPNIQNPDPAVYQLRDSKSSDKSVCLFTDFDSQTNVSQSKDSDVYITDKTVLDMRSMDFKSNSAVAWSNKSDFACANAFNNSIIPEDTFFPSPESSCDVKLVEKSFETDTNLNFQNLSVIGFRILLLKVAGFNLLMTLRLWSS

SEQ ID NO: 31 - protein, 5 aa, Homo sapiens
SGHAT

SEQ ID NO: 32 - protein, 6 aa, Homo sapiens
FQNNGV

SEQ ID NO: 33 - protein, 13 aa, Homo sapiens
CASSYTNQGEAFF

SEQ ID NO: 34 - protein, 132 aa, Homo sapiens
MGTRLLCWAALCLLGAELTEAGVAQSPRYKIIEKRQSVAFWCNPISGHATLYWYQQILGQGPKLLIQFQNNGVVDDSQLPKDRFSAERLKGVDSTLKIQPAKLEDSAVYLCASSYTNQGEAFFGQGTRLTVV

SEQ ID NO: 35 - protein, 177 aa, Homo sapiens
EDLNKVFPPEVAVFEPSEAEISHTQKATLVCLATGFFPDHVELSWWVNGKEVHSGVSTDPQPLKEQPALNDSRYCLSSRLRVSATFWQNPRNHFRCQVQFYGLSENDEWTQDRAKPVTQIVSAEAWGRADCGFTSVSYQQGVLSATILYEILLGKATLYAVLVSALVLMAMVKRKDF

SEQ ID NO: 36 - protein, 309 aa, Homo sapiens
MGTRLLCWAALCLLGAELTEAGVAQSPRYKIIEKRQSVAFWCNPISGHATLYWYQQILGQGPKLLIQFQNNGVVDDSQLPKDRFSAERLKGVDSTLKIQPAKLEDSAVYLCASSYTNQGEAFFGQGTRLTVVEDLNKVFPPEVAVFEPSEAEISHTQKATLVCLATGFFPDHVELSWWVNGKEVHSGVSTDPQPLKEQPALNDSRYCLSSRLRVSATFWQNPRNHFRCQVQFYGLSENDEWTQDRAKPVTQIVSAEAWGRADCGFTSVSYQQGVLSATILYEILLGKATLYAVLVSALVLMAMVKRKDF

SEQ ID NO: 37 - protein, 6 aa, Homo sapiens
DRGSQS

SEQ ID NO: 38 - protein, 2 aa, Homo sapiens
IY

SEQ ID NO: 39 - protein, 13 aa, Homo sapiens
CAVLNQAGTALIF

SEQ ID NO: 40 - protein, 132 aa, Homo sapiens
MKSLRVLLVILWLQLSWVWSQQKEVEQNSGPLSVPEGAIASLNCTYSDRGSQSFFWYRQYSGKSPELIMSIYSNGDKEDGRFTAQLNKASQYVSLLIRDSQPSDSATYLCAVLNQAGTALIFGKGTTLSVSS

SEQ ID NO: 41 - protein, 141 aa, Homo sapiens; identical to SEQ ID NO: 5

SEQ ID NO: 42 - protein, 273 aa, Homo sapiens
MKSLRVLLVILWLQLSWVWSQQKEVEQNSGPLSVPEGAIASLNCTYSDRGSQSFFWYRQYSGKSPELIMSIYSNGDKEDGRFTAQLNKASQYVSLLIRDSQPSDSATYLCAVLNQAGTALIFGKGTTLSVSSNIQNPDPAVYQLRDSKSSDKSVCLFTDFDSQTNVSQSKDSDVYITDKTVLDMRSMDFKSNSAVAWSNKSDFACANAFNNSIIPEDTFFPSPESSCDVKLVEKSFETDTNLNFQNLSVIGFRILLLKVAGFNLLMTLRLWSS

SEQ ID NO: 43 - protein, 5 aa, Homo sapiens
SGDLS

SEQ ID NO: 44 - protein, 6 aa, Homo sapiens
YYNGEE

SEQ ID NO: 45 - protein, 17 aa, Homo sapiens
CASSAETGPWLGNEQFF

SEQ ID NO: 46 - protein, 135 aa, Homo sapiens
MGFRLLCCVAFCLLGAGPVDSGVTQTPKHLITATGQRVTLRCSPRSGDLSVYWYQQSLDQGLQFLIQYYNGEERAKGNILERFSAQQFPDLHSELNLSSLELGDSALYFCASSAETGPWLGNEQFFGPGTRLTVL

SEQ ID NO: 47 - protein, 179 aa, Homo sapiens; identical to SEQ ID NO: 11

SEQ ID NO: 48 - protein, 314 aa, Homo sapiens
MGFRLLCCVAFCLLGAGPVDSGVTQTPKHLITATGQRVTLRCSPRSGDLSVYWYQQSLDQGLQFLIQYYNGEERAKGNILERFSAQQFPDLHSELNLSSLELGDSALYFCASSAETGPWLGNEQFFGPGTRLTVLEDLKNVFPPEVAVFEPSEAEISHTQKATLVCLATGFYPDHVELSWWVNGKEVHSGVSTDPQPLKEQPALNDSRYCLSSRLRVSATFWQNPRNHFRCQVQFYGLSENDEWTQDRAKPVTQIVSAEAWGRADCGFTSESYQQGVLSATILYEILLGKATLYAVLVSALVLMAMVKRKDSRG

SEQ ID NO: 49 - protein, 7 aa, Homo sapiens
TSESDYY

SEQ ID NO: 50 - protein, 4 aa, Homo sapiens
QEAY

SEQ ID NO: 51 - protein, 15 aa, Homo sapiens
CAYRWAQGGSEKLVF

SEQ ID NO: 52 - protein, 136 aa, Homo sapiens
MACPGFLWALVISTCLEFSMAQTVTQSQPEMSVQEAETVTLSCTYDTSESDYYLFWYKQPPSRQMILVIRQEAYKQQNATENRFSVNFQKAAKSFSLKISDSQLGDAAMYFCAYRWAQGGSEKLVFGKGTKLTVNP

SEQ ID NO: 53 - protein, 141 aa, Homo sapiens
YIQKPDPAVYQLRDSKSSDKSVCLFTDFDSQTNVSQSKDSDVYITDKTVLDMRSMDFKSNSAVAWSNKSDFACANAFNNSIIPEDTFFPSPESSCDVKLVEKSFETDTNLNFQNLSVIGFRILLLKVAGFNLLMTLRLWSS

SEQ ID NO: 54 - protein, 277 aa, Homo sapiens
MACPGFLWALVISTCLEFSMAQTVTQSQPEMSVQEAETVTLSCTYDTSESDYYLFWYKQPPSRQMILVIRQEAYKQQNATENRFSVNFQKAAKSFSLKISDSQLGDAAMYFCAYRWAQGGSEKLVFGKGTKLTVNPYIQKPDPAVYQLRDSKSSDKSVCLFTDFDSQTNVSQSKDSDVYITDKTVLDMRSMDFKSNSAVAWSNKSDFACANAFNNSIIPEDTFFPSPESSCDVKLVEKSFETDTNLNFQNLSVIGFRILLLKVAGFNLLMTLRLWSS

SEQ ID NO: 55 - protein, 5 aa, Homo sapiens
MGHDK

SEQ ID NO: 56 - protein, 6 aa, Homo sapiens
SYGVNS

SEQ ID NO: 57 - protein, 16 aa, Homo sapiens
CATELWSSGGTGELFF

SEQ ID NO: 58 - protein, 134 aa, Homo sapiens
MTIRLLCYMGFYFLGAGLMEADIYQTPRYLVIGTGKKITLECSQTMGHDKMYWYQQDPGMELHLIHYSYGVNSTEKGDLSSESTVSRIRTEHFPLTLESARPSHTSQYLCATELWSSGGTGELFFGEGSRLTVL

SEQ ID NO: 59 - protein, 179 aa, Homo sapiens; identical to SEQ ID NO: 11

SEQ ID NO: 60 - protein, 313 aa, Homo sapiens
MTIRLLCYMGFYFLGAGLMEADIYQTPRYLVIGTGKKITLECSQTMGHDKMYWYQQDPGMELHLIHYSYGVNSTEKGDLSSESTVSRIRTEHFPLTLESARPSHTSQYLCATELWSSGGTGELFFGEGSRLTVLEDLKNVFPPEVAVFEPSEAEISHTQKATLVCLATGFYPDHVELSWWVNGKEVHSGVSTDPQPLKEQPALNDSRYCLSSRLRVSATFWQNPRNHFRCQVQFYGLSENDEWTQDRAKPVTQIVSAEAWGRADCGFTSESYQQGVLSATILYEILLGKATLYAVLVSALVLMAMVKRKDSRG

SEQ ID NO: 61 - protein, 6 aa, Homo sapiens
DRGSQS

SEQ ID NO: 62 - protein, 2 aa, Homo sapiens
IY

SEQ ID NO: 63 - protein, 13 aa, Homo sapiens
CAVGPSGTYKYIF

SEQ ID NO: 64 - protein, 132 aa, Homo sapiens
MKSLRVLLVILWLQLSWVWSQQKEVEQNSGPLSVPEGAIASLNCTYSDRGSQSFFWYRQYSGKSPELIMSIYSNGDKEDGRFTAQLNKASQYVSLLIRDSQPSDSATYLCAVGPSGTYKYIFGTGTRLKVLA

SEQ ID NO: 65 - protein, 141 aa, Homo sapiens; identical to SEQ ID NO: 5

SEQ ID NO: 66 - protein, 273 aa, Homo sapiens
MKSLRVLLVILWLQLSWVWSQQKEVEQNSGPLSVPEGAIASLNCTYSDRGSQSFFWYRQYSGKSPELIMSIYSNGDKEDGRFTAQLNKASQYVSLLIRDSQPSDSATYLCAVGPSGTYKYIFGTGTRLKVLANIQNPDPAVYQLRDSKSSDKSVCLFTDFDSQTNVSQSKDSDVYITDKTVLDMRSMDFKSNSAVAWSNKSDFACANAFNNSIIPEDTFFPSPESSCDVKLVEKSFETDTNLNFQNLSVIGFRILLLKVAGFNLLMTLRLWSS

SEQ ID NO: 67 - protein, 5 aa, Homo sapiens
MNHEY

SEQ ID NO: 68 - protein, 6 aa, Homo sapiens
SMNVEV

SEQ ID NO: 69 - protein, 14 aa, Homo sapiens
CASSPGGSGNEQFF

SEQ ID NO: 70 - protein, 132 aa, Homo sapiens
MGPQLLGYVVLCLLGAGPLEAQVTQNPRYLITVTGKKLTVTCSQNMNHEYMSWYRQDPGLGLRQIYYSMNVEVTDKGDVPEGYKVSRKEKRNFPLILESPSPNQTSLYFCASSPGGSGNEQFFGPGTRLTVL

SEQ ID NO: 71 - protein, 179 aa, Homo sapiens; identical to SEQ ID NO: 11

SEQ ID NO: 72 - protein, 311 aa, Homo sapiens
MGPQLLGYVVLCLLGAGPLEAQVTQNPRYLITVTGKKLTVTCSQNMNHEYMSWYRQDPGLGLRQIYYSMNVEVTDKGDVPEGYKVSRKEKRNFPLILESPSPNQTSLYFCASSPGGSGNEQFFGPGTRLTVLEDLKNVFPPEVAVFEPSEAEISHTQKATLVCLATGFYPDHVELSWWVNGKEVHSGVSTDPQPLKEQPALNDSRYCLSSRLRVSATFWQNPRNHFRCQVQFYGLSENDEWTQDRAKPVTQIVSAEAWGRADCGFTSESYQQGVLSATILYEILLGKATLYAVLVSALVLMAMVKRKDSRG

SEQ ID NO: 73 - protein, 6 aa, Homo sapiens
DRGSQS

SEQ ID NO: 74 - protein, 2 aa, Homo sapiens
IY

SEQ ID NO: 75 - protein, 14 aa, Homo sapiens
CAVVSGGGADGLTF

SEQ ID NO: 76 - protein, 133 aa, Homo sapiens
MKSLRVLLVILWLQLSWVWSQQKEVEQNSGPLSVPEGAIASLNCTYSDRGSQSFFWYRQYSGKSPELIMFIYSNGDKEDGRFTAQLNKASQYVSLLIRDSQPSDSATYLCAVVSGGGADGLTFGKGTHLIIQP

SEQ ID NO: 77 - protein, 141 aa, Homo sapiens; identical to SEQ ID NO: 53

SEQ ID NO: 78 - protein, 274 aa, Homo sapiens
MKSLRVLLVILWLQLSWVWSQQKEVEQNSGPLSVPEGAIASLNCTYSDRGSQSFFWYRQYSGKSPELIMFIYSNGDKEDGRFTAQLNKASQYVSLLIRDSQPSDSATYLCAVVSGGGADGLTFGKGTHLIIQPYIQKPDPAVYQLRDSKSSDKSVCLFTDFDSQTNVSQSKDSDVYITDKTVLDMRSMDFKSNSAVAWSNKSDFACANAFNNSIIPEDTFFPSPESSCDVKLVEKSFETDTNLNFQNLSVIGFRILLLKVAGFNLLMTLRLWSS

SEQ ID NO: 79 - protein, 5 aa, Homo sapiens
PRHDT

SEQ ID NO: 80 - protein, 6 aa, Homo sapiens
FYEKMQ

SEQ ID NO: 81 - protein, 14 aa, Homo sapiens
CASSLGRGGQPQHF

SEQ ID NO: 82 - protein, 142 aa, Homo sapiens
MLSPDLPDSAWNTRLLCHVMLCLLGAVSVAAGVIQSPRHLIKEKRETATLKCYPIPRHDTVYWYQQGPGQDPQFLISFYEKMQSDKGSIPDRFSAQQFSDYHSELNMSSLELGDSALYFCASSLGRGGQPQHFGDGTRLSIL

SEQ ID NO: 83 - protein, 177 aa, Homo sapiens; identical to SEQ ID NO: 35

SEQ ID NO: 84 - protein, 319 aa, Homo sapiens
MLSPDLPDSAWNTRLLCHVMLCLLGAVSVAAGVIQSPRHLIKEKRETATLKCYPIPRHDTVYWYQQGPGQDPQFLISFYEKMQSDKGSIPDRFSAQQFSDYHSELNMSSLELGDSALYFCASSLGRGGQPQHFGDGTRLSILEDLNKVFPPEVAVFEPSEAEISHTQKATLVCLATGFFPDHVELSWWVNGKEVHSGVSTDPQPLKEQPALNDSRYCLSSRLRVSATFWQNPRNHFRCQVQFYGLSENDEWTQDRAKPVTQIVSAEAWGRADCGFTSVSYQQGVLSATILYEILLGKATLYAVLVSALVLMAMVKRKDF

SEQ ID NO: 85 - protein, 6 aa, Homo sapiens
DSAIYN

SEQ ID NO: 86 - protein, 3 aa, Homo sapiens
IQS

SEQ ID NO: 87 - protein, 15 aa, Homo sapiens
CAVRPTSGGSYIPTF

SEQ ID NO: 88 - protein, 133 aa, Homo sapiens
METLLGLLILWLQLQWVSSKQEVTQIPAALSVPEGENLVLNCSFTDSAIYNLQWFRQDPGKGLTSLLLIQSSQREQTSGRLNASLDKSSGRSTLYIAASQPGDSATYLCAVRPTSGGSYIPTFGRGTSLIVHP

SEQ ID NO: 89 - protein, 141 aa, Homo sapiens
YIQNPDPAVYQLRDSKSSDKSVCLFTDFDSQTNVSQSKDSDVYITDKTVLDMRSMDFKSNSAVAWSNKSDFACANAFNNSIIPEDTFFPSPESSCDVKLVEKSFETDTNLNFQNLSVIGFRILLLKVAGFNLLMTLRLWSS

SEQ ID NO: 90 - protein, 274 aa, Homo sapiens
METLLGLLILWLQLQWVSSKQEVTQIPAALSVPEGENLVLNCSFTDSAIYNLQWFRQDPGKGLTSLLLIQSSQREQTSGRLNASLDKSSGRSTLYIAASQPGDSATYLCAVRPTSGGSYIPTFGRGTSLIVHPYIQNPDPAVYQLRDSKSSDKSVCLFTDFDSQTNVSQSKDSDVYITDKTVLDMRSMDFKSNSAVAWSNKSDFACANAFNNSIIPEDTFFPSPESSCDVKLVEKSFETDTNLNFQNLSVIGFRILLLKVAGFNLLMTLRLWSS

SEQ ID NO: 91 - protein, 5 aa, Homo sapiens
MNHEY

SEQ ID NO: 92 - protein, 6 aa, Homo sapiens
SVGAGI

SEQ ID NO: 93 - protein, 14 aa, Homo sapiens
CASSYVGNTGELFF

SEQ ID NO: 94 - protein, 132 aa, Homo sapiens
MSIGLLCCAALSLLWAGPVNAGVTQTPKFQVLKTGQSMTLQCAQDMNHEYMSWYRQDPGMGLRLIHYSVGAGITDQGEVPNGYNVSRSTTEDFPLRLLSAAPSQTSVYFCASSYVGNTGELFFGEGSRLTVL

SEQ ID NO: 95 - protein, 179 aa, Homo sapiens; identical to SEQ ID NO: 11

SEQ ID NO: 96 - protein, 311 aa, Homo sapiens
MSIGLLCCAALSLLWAGPVNAGVTQTPKFQVLKTGQSMTLQCAQDMNHEYMSWYRQDPGMGLRLIHYSVGAGITDQGEVPNGYNVSRSTTEDFPLRLLSAAPSQTSVYFCASSYVGNTGELFFGEGSRLTVLEDLKNVFPPEVAVFEPSEAEISHTQKATLVCLATGFYPDHVELSWWVNGKEVHSGVSTDPQPLKEQPALNDSRYCLSSRLRVSATFWQNPRNHFRCQVQFYGLSENDEWTQDRAKPVTQIVSAEAWGRADCGFTSESYQQGVLSATILYEILLGKATLYAVLVSALVLMAMVKRKDSRG

SEQ ID NO: 97 - protein, 9 aa, Homo sapiens
SLLQHLIGL

SEQ ID NO: 98 - protein, 9 aa, Homo sapiens
ALLQHLIGL

SEQ ID NO: 99 - protein, 9 aa, Homo sapiens
SALQHLIGL

SEQ ID NO: 100 - protein, 9 aa, Homo sapiens
SLAQHLIGL

SEQ ID NO: 101 - protein, 9 aa, Homo sapiens
SLLAHLIGL

SEQ ID NO: 102 - protein, 9 aa, Homo sapiens
SLLQALIGL

SEQ ID NO: 103 - protein, 9 aa, Homo sapiens
SLLQHAIGL

SEQ ID NO: 104 - protein, 9 aa, Homo sapiens
SLLQHLAGL

SEQ ID NO: 105 - protein, 9 aa, Homo sapiens
SLLQHLIAL

SEQ ID NO: 106 - protein, 9 aa, Homo sapiens
SLLQHLIGA

SEQ ID NO: 107 - protein, 9 aa, Homo sapiens
TLLQHLIGL

SEQ ID NO: 108 - protein, 9 aa, Homo sapiens
STLQHLIGL

SEQ ID NO: 109 - protein, 9 aa, Homo sapiens
SLTQHLIGL

SEQ ID NO: 110 - protein, 9 aa, Homo sapiens
SLLTHLIGL

SEQ ID NO: 111 - protein, 9 aa, Homo sapiens
SLLQTLIGL

SEQ ID NO: 112 - protein, 9 aa, Homo sapiens
SLLQHTIGL

SEQ ID NO: 113 - protein, 9 aa, Homo sapiens
SLLQHLTGL

SEQ ID NO: 114 - protein, 9 aa, Homo sapiens
SLLQHLITL

SEQ ID NO: 115 - protein, 9 aa, Homo sapiens
SLLQHLIGT

SEQ ID NO: 116 - protein, 9 aa, Homo sapiens
SILQTLILV

SEQ ID NO: 117 - protein, 9 aa, Homo sapiens
SLIEHLQGL

SEQ ID NO: 118 - protein, 9 aa, Homo sapiens
SLIQHLEEI

SEQ ID NO: 119 - protein, 9 aa, Homo sapiens
SLLKNLIYL

SEQ ID NO: 120 - protein, 9 aa, Homo sapiens
SLLNHLPYL

SEQ ID NO: 121 - protein, 9 aa, Homo sapiens
SLLQHVLLL

SEQ ID NO: 122 - protein, 9 aa, Homo sapiens
SLLQKQIML

SEQ ID NO: 123 - protein, 9 aa, Homo sapiens
SLSQELVGV

SEQ ID NO: 124 - protein, 9 aa, Homo sapiens
SVLGALIGV

SEQ ID NO: 125 - protein, 9 aa, Homo sapiens
VLLHHQIGL

SEQ ID NO: 126 - protein, 9 aa, Homo sapiens
SLLMWITQV

SEQ ID NO: 127 - protein, 6 aa, Homo sapiens
SSNFYA

SEQ ID NO: 128 - protein, 3 aa, Homo sapiens
MTL

SEQ ID NO: 129 - protein, 11 aa, Homo sapiens
CALYNNNDMRF

SEQ ID NO: 130 - protein, 132 aa, Homo sapiens
MEKNPLAAPLLILWFHLDCVSSILNVEQSPQSLHVQEGDSTNFTCSFPSSNFYALHWYRKETAKSPEALFVMTLNGDEKKKGRISATLNTKEGYSYLYIKGSQPEDSATYLCALYNNNDMRFGAGTRLTVKP

SEQ ID NO: 131 - protein, 141 aa, Homo sapiens; identical to SEQ ID NO: 5

SEQ ID NO: 132 - protein, 273 aa, Homo sapiens
MEKNPLAAPLLILWFHLDCVSSILNVEQSPQSLHVQEGDSTNFTCSFPSSNFYALHWYRKETAKSPEALFVMTLNGDEKKKGRISATLNTKEGYSYLYIKGSQPEDSATYLCALYNNNDMRFGAGTRLTVKPNIQNPDPAVYQLRDSKSSDKSVCLFTDFDSQTNVSQSKDSDVYITDKTVLDMRSMDFKSNSAVAWSNKSDFACANAFNNSIIPEDTFFPSPESSCDVKLVEKSFETDTNLNFQNLSVIGFRILLLKVAGFNLLMTLRLWSS

SEQ ID NO: 133 - protein, 5 aa, Homo sapiens
SGHNS

SEQ ID NO: 134 - protein, 6 aa, Homo sapiens
FNNNVP

SEQ ID NO: 135 - protein, 13 aa, Homo sapiens
CASSPGSTDTQYF

SEQ ID NO: 136 - protein, 132 aa, Homo sapiens
MDSWTFCCVSLCILVAKHTDAGVIQSPRHEVTEMGQEVTLRCKPISGHNSLFWYRETMMRGLELLIYFNNNVPIDDSGMPEDRFSAKMPNASFSTLKIQPSEPRDSAVYFCASSPGSTDTQYFGPGTRLTVL

SEQ ID NO: 137 - protein, 179 aa, Homo sapiens; identical to SEQ ID NO: 11

SEQ ID NO: 138 - protein, 311 aa, Homo sapiens
MDSWTFCCVSLCILVAKHTDAGVIQSPRHEVTEMGQEVTLRCKPISGHNSLFWYRETMMRGLELLIYFNNNVPIDDSGMPEDRFSAKMPNASFSTLKIQPSEPRDSAVYFCASSPGSTDTQYFGPGTRLTVLEDLKNVFPPEVAVFEPSEAEISHTQKATLVCLATGFYPDHVELSWWVNGKEVHSGVSTDPQPLKEQPALNDSRYCLSSRLRVSATFWQNPRNHFRCQVQFYGLSENDEWTQDRAKPVTQIVSAEAWGRADCGFTSESYQQGVLSATILYEILLGKATLYAVLVSALVLMAMVKRKDSRG

SEQ ID NO: 139 - protein, 9 aa, Homo sapiens
LLLVHLIPV

SEQ ID NO: 140 - protein, 9 aa, Homo sapiens
IILRHLIEI

SEQ ID NO: 141 - protein, 9 aa, Homo sapiens
KILLHLIHI

SEQ ID NO: 142 - protein, 9 aa, Homo sapiens
KVLPHLIPL

SEQ ID NO: 143 - protein, 9 aa, Homo sapiens
SALVHLIPV

SEQ ID NO: 144 - protein, 9 aa, Homo sapiens
NALVHLIEV

SEQ ID NO: 145 - protein, 9 aa, Homo sapiens
VALGHLIGI

SEQ ID NO: 146 - protein, 9 aa, Homo sapiens
NALVHLIEI

SEQ ID NO: 147 - protein, 9 aa, Homo sapiens
WALGHLIGI

SEQ ID NO: 148 - protein, 9 aa, Homo sapiens
QALEHLIYI

SEQ ID NO: 149 - protein, 9 aa, Homo sapiens
ISLAHLILV

SEQ ID NO: 150 - protein, 9 aa, Homo sapiens
ETLDHLISL

SEQ ID NO: 151 - protein, 9 aa, Homo sapiens
ALLSHLICR

SEQ ID NO: 152 - protein, 9 aa, Homo sapiens
KELRHLIEV

SEQ ID NO: 153 - protein, 9 aa, Homo sapiens
IALVHLIMV

SEQ ID NO: 154 - protein, 9 aa, Homo sapiens
CWLCHLIKL

SEQ ID NO: 155 - protein, 9 aa, Homo sapiens
GKLTHLIPV

SEQ ID NO: 156 - protein, 9 aa, Homo sapiens
HLLMHLIGS

SEQ ID NO: 157 - protein, 9 aa, Homo sapiens
TQLDHLIPG

SEQ ID NO: 158 - protein, 9 aa, Homo sapiens
QDLWHLIKL

SEQ ID NO: 159 - protein, 9 aa, Homo sapiens
IALKHLIPT

SEQ ID NO: 160 - protein, 9 aa, Homo sapiens
IALKHLILT

SEQ ID NO: 161 - protein, 9 aa, Homo sapiens
LQLIHLINV

SEQ ID NO: 162 - protein, 9 aa, Homo sapiens
SQLVHLIYV

SEQ ID NO: 163 - protein, 9 aa, Homo sapiens
CLLPHLIQH

SEQ ID NO: 164 - protein, 9 aa, Homo sapiens
MVLVHLIHS

SEQ ID NO: 165 - protein, 9 aa, Homo sapiens
SDLFHLIGV

SEQ ID NO: 166 - protein, 9 aa, Homo sapiens
KLLFHLIQS

SEQ ID NO: 167 - protein, 9 aa, Homo sapiens
KLLLHLIQS

SEQ ID NO: 168 - protein, 9 aa, Homo sapiens
SFLVHLIGL

SEQ ID NO: 169 - protein, 9 aa, Homo sapiens
YGLKHLISV

SEQ ID NO: 170 - protein, 9 aa, Homo sapiens
SELPHLIGI

SEQ ID NO: 171 - protein, 9 aa, Homo sapiens
YALSHLIHA

SEQ ID NO: 172 - protein, 9 aa, Homo sapiens
TLLGHLISK

SEQ ID NO: 173 - protein, 9 aa, Homo sapiens
SQLSHLIAM

SEQ ID NO: 174 - protein, 9 aa, Homo sapiens
FFLVHLICM

SEQ ID NO: 175 - protein, 9 aa, Homo sapiens
VSLHHLINA

SEQ ID NO: 176 - protein, 9 aa, Homo sapiens
IMLIHLIRL

SEQ ID NO: 177 - protein, 9 aa, Homo sapiens
ITLIHLIRL

SEQ ID NO: 178 - protein, 9 aa, Homo sapiens
SELFHLIPL

SEQ ID NO: 179 - protein, 9 aa, Homo sapiens
SVLFHLIPL

SEQ ID NO: 180 - protein, 9 aa, Homo sapiens
AQLAHLILS

SEQ ID NO: 181 - protein, 9 aa, Homo sapiens
FLLGHLIPR

SEQ ID NO: 182 - protein, 9 aa, Homo sapiens
MLLGHLIFF

SEQ ID NO: 183 - protein, 9 aa, Homo sapiens
VLLFHLIEE

SEQ ID NO: 184 - protein, 9 aa, Homo sapiens
VFLRHLITL

SEQ ID NO: 185 - protein, 9 aa, Homo sapiens
TLLDHLIFK

SEQ ID NO: 186 - protein, 9 aa, Homo sapiens
SVLVHLIPA

SEQ ID NO: 187 - protein, 9 aa, Homo sapiens
AKLEHLIYL

SEQ ID NO: 188 - protein, 9 aa, Homo sapiens
SLLPHLILS

SEQ ID NO: 189 - protein, 9 aa, Homo sapiens
SILGHLICS

SEQ ID NO: 190 - protein, 9 aa, Homo sapiens
QSLEHLIYI

SEQ ID NO: 191 - protein, 9 aa, Homo sapiens
YILNHLINP

SEQ ID NO: 192 - protein, 9 aa, Homo sapiens
YKLLHLIWI

SEQ ID NO: 193 - protein, 9 aa, Homo sapiens
KLLCHLIEH

SEQ ID NO: 194 - protein, 9 aa, Homo sapiens
ALLDHLITH

SEQ ID NO: 195 - protein, 9 aa, Homo sapiens
FMLSHLIQH

SEQ ID NO: 196 - protein, 7 aa, Homo sapiens
MTLNGDE

SEQ ID NO: 197 - protein, 6 aa, Homo sapiens
IYSNGD

SEQ ID NO: 198 - protein, 6 aa, Homo sapiens
TYSSGN

SEQ ID NO: 199 - protein, 6 aa, Homo sapiens
IYSNGD

SEQ ID NO: 200 - protein, 7 aa, Homo sapiens
QEAYKQQ

SEQ ID NO: 201 - protein, 6 aa, Homo sapiens
IYSNGD

SEQ ID NO: 202 - protein, 6 aa, Homo sapiens
IYSNGD

SEQ ID NO: 203 - protein, 7 aa, Homo sapiens
IQSSQRE

SEQ ID NO: 204 - protein, 7 aa, Homo sapiens
MTLNGDE